European Patent Specification EP 3 519 579 B1, published November 5, 2025. Title: Process to Prepare Elongated 2-Ketoacids and C5-C10 Compounds Therefrom via Genetic Modifications to Microbial Metabolic Pathways. Applicant: The Dow Chemical Company Sanghani, Paresh Greenwalt, Scott Bhosale, Prakash Shiue, Eric. The sequence listing filed with the application follows.

SEQUENCE LISTING (37 sequences)

SEQ ID NO: 1 - protein, 466 aa, Escherichia coli
MAKTLYEKLFDAHVVYEAENETPLLYIDRHLVHEVTSPQAFDGLRAHGRPVRQPGKTFATMDHNVSTQTKDINACGEMARIQMQELIKNCKEFGVELYDLNHPYQGIVHVMGPEQGVTLPGMTIVCGDSHTATHGAFGALAFGIGTSEVEHVLATQTLKQGRAKTMKIEVQGKAAPGITAKDIVLAIIGKTGSAGGTGHVVEFCGEAIRDLSMEGRMTLCNMAIEMGAKAGLVAPDETTFNYVKGRLHAPKGKDFDDAVAYWKTLQTDEGATFDTVVTLQAEEISPQVTWGTNPGQVISVNDNIPDPASFADPVERASAEKALAYMGLKPGIPLTEVAIDKVFIGSCTNSRIEDLRAAAEIAKGRKVAPGVQALVVPGSGPVKAQAEAEGLDKIFIEAGFEWRLPGCSMCLAMNNDRLNPGERCASTSNRNFEGRQGRGGRTHLVSPAMAAAAAVTGHFADIRNIK

SEQ ID NO: 2 - protein, 201 aa, Escherichia coli
MAEKFIKHTGLVVPLDAANVDTDAIIPKQFLQKVTRTGFGAHLFNDWRFLDEKGQQPNPDFVLNFPQYQGASILLARENFGCGSSREHAPWALTDYGFKVVIAPSFADIFYGNSFNNQLLPVKLSDAEVDELFALVKANPGIHFDVDLEAQEVKAGEKTYRFTIDAFRRHCMMNGLDSIGLTLQHDDAIAAYEAKQPAFMN

SEQ ID NO: 3 - protein, 466 aa, Artificial Sequence
  Synthesized - Modified LeuC (V35A)
MAKTLYEKLFDAHVVYEAENETPLLYIDRHLVHEATSPQAFDGLRAHGRPVRQPGKTFATMDHNVSTQTKDINACGEMARIQMQELIKNCKEFGVELYDLNHPYQGIVHVMGPEQGVTLPGMTIVCGDSHTATHGAFGALAFGIGTSEVEHVLATQTLKQGRAKTMKIEVQGKAAPGITAKDIVLAIIGKTGSAGGTGHVVEFCGEAIRDLSMEGRMTLCNMAIEMGAKAGLVAPDETTFNYVKGRLHAPKGKDFDDAVAYWKTLQTDEGATFDTVVTLQAEEISPQVTWGTNPGQVISVNDNIPDPASFADPVERASAEKALAYMGLKPGIPLTEVAIDKVFIGSCTNSRIEDLRAAAEIAKGRKVAPGVQALVVPGSGPVKAQAEAEGLDKIFIEAGFEWRLPGCSMCLAMNNDRLNPGERCASTSNRNFEGRQGRGGRTHLVSPAMAAAAAVTGHFADIRNIK

SEQ ID NO: 4 - protein, 466 aa, Artificial Sequence
  Synthesized - Modified LeuC (V35G)
MAKTLYEKLFDAHVVYEAENETPLLYIDRHLVHEGTSPQAFDGLRAHGRPVRQPGKTFATMDHNVSTQTKDINACGEMARIQMQELIKNCKEFGVELYDLNHPYQGIVHVMGPEQGVTLPGMTIVCGDSHTATHGAFGALAFGIGTSEVEHVLATQTLKQGRAKTMKIEVQGKAAPGITAKDIVLAIIGKTGSAGGTGHVVEFCGEAIRDLSMEGRMTLCNMAIEMGAKAGLVAPDETTFNYVKGRLHAPKGKDFDDAVAYWKTLQTDEGATFDTVVTLQAEEISPQVTWGTNPGQVISVNDNIPDPASFADPVERASAEKALAYMGLKPGIPLTEVAIDKVFIGSCTNSRIEDLRAAAEIAKGRKVAPGVQALVVPGSGPVKAQAEAEGLDKIFIEAGFEWRLPGCSMCLAMNNDRLNPGERCASTSNRNFEGRQGRGGRTHLVSPAMAAAAAVTGHFADIRNIK

SEQ ID NO: 5 - protein, 466 aa, Artificial Sequence
  Synthezied - Modified LeuC (L411A)
MAKTLYEKLFDAHVVYEAENETPLLYIDRHLVHEVTSPQAFDGLRAHGRPVRQPGKTFATMDHNVSTQTKDINACGEMARIQMQELIKNCKEFGVELYDLNHPYQGIVHVMGPEQGVTLPGMTIVCGDSHTATHGAFGALAFGIGTSEVEHVLATQTLKQGRAKTMKIEVQGKAAPGITAKDIVLAIIGKTGSAGGTGHVVEFCGEAIRDLSMEGRMTLCNMAIEMGAKAGLVAPDETTFNYVKGRLHAPKGKDFDDAVAYWKTLQTDEGATFDTVVTLQAEEISPQVTWGTNPGQVISVNDNIPDPASFADPVERASAEKALAYMGLKPGIPLTEVAIDKVFIGSCTNSRIEDLRAAAEIAKGRKVAPGVQALVVPGSGPVKAQAEAEGLDKIFIEAGFEWRLPGCSMCAAMNNDRLNPGERCASTSNRNFEGRQGRGGRTHLVSPAMAAAAAVTGHFADIRNIK

SEQ ID NO: 6 - protein, 466 aa, Artificial Sequence
  Synthesized - Modified LeuC (L411G)
MAKTLYEKLFDAHVVYEAENETPLLYIDRHLVHEVTSPQAFDGLRAHGRPVRQPGKTFATMDHNVSTQTKDINACGEMARIQMQELIKNCKEFGVELYDLNHPYQGIVHVMGPEQGVTLPGMTIVCGDSHTATHGAFGALAFGIGTSEVEHVLATQTLKQGRAKTMKIEVQGKAAPGITAKDIVLAIIGKTGSAGGTGHVVEFCGEAIRDLSMEGRMTLCNMAIEMGAKAGLVAPDETTFNYVKGRLHAPKGKDFDDAVAYWKTLQTDEGATFDTVVTLQAEEISPQVTWGTNPGQVISVNDNIPDPASFADPVERASAEKALAYMGLKPGIPLTEVAIDKVFIGSCTNSRIEDLRAAAEIAKGRKVAPGVQALVVPGSGPVKAQAEAEGLDKIFIEAGFEWRLPGCSMCGAMNNDRLNPGERCASTSNRNFEGRQGRGGRTHLVSPAMAAAAAVTGHFADIRNIK

SEQ ID NO: 7 - protein, 466 aa, Artificial Sequence
  Synthesized - Modified LeuC (L411V)
MAKTLYEKLFDAHVVYEAENETPLLYIDRHLVHEVTSPQAFDGLRAHGRPVRQPGKTFATMDHNVSTQTKDINACGEMARIQMQELIKNCKEFGVELYDLNHPYQGIVHVMGPEQGVTLPGMTIVCGDSHTATHGAFGALAFGIGTSEVEHVLATQTLKQGRAKTMKIEVQGKAAPGITAKDIVLAIIGKTGSAGGTGHVVEFCGEAIRDLSMEGRMTLCNMAIEMGAKAGLVAPDETTFNYVKGRLHAPKGKDFDDAVAYWKTLQTDEGATFDTVVTLQAEEISPQVTWGTNPGQVISVNDNIPDPASFADPVERASAEKALAYMGLKPGIPLTEVAIDKVFIGSCTNSRIEDLRAAAEIAKGRKVAPGVQALVVPGSGPVKAQAEAEGLDKIFIEAGFEWRLPGCSMCVAMNNDRLNPGERCASTSNRNFEGRQGRGGRTHLVSPAMAAAAAVTGHFADIRNIK

SEQ ID NO: 8 - protein, 466 aa, Artificial Sequence
  Synthesized - Modified LeuC (V35A L411A)
MAKTLYEKLFDAHVVYEAENETPLLYIDRHLVHEATSPQAFDGLRAHGRPVRQPGKTFATMDHNVSTQTKDINACGEMARIQMQELIKNCKEFGVELYDLNHPYQGIVHVMGPEQGVTLPGMTIVCGDSHTATHGAFGALAFGIGTSEVEHVLATQTLKQGRAKTMKIEVQGKAAPGITAKDIVLAIIGKTGSAGGTGHVVEFCGEAIRDLSMEGRMTLCNMAIEMGAKAGLVAPDETTFNYVKGRLHAPKGKDFDDAVAYWKTLQTDEGATFDTVVTLQAEEISPQVTWGTNPGQVISVNDNIPDPASFADPVERASAEKALAYMGLKPGIPLTEVAIDKVFIGSCTNSRIEDLRAAAEIAKGRKVAPGVQALVVPGSGPVKAQAEAEGLDKIFIEAGFEWRLPGCSMCAAMNNDRLNPGERCASTSNRNFEGRQGRGGRTHLVSPAMAAAAAVTGHFADIRNIK

SEQ ID NO: 9 - protein, 466 aa, Artificial Sequence
  Synthesized - Modified LeuC (V35A L411G)
MAKTLYEKLFDAHVVYEAENETPLLYIDRHLVHEATSPQAFDGLRAHGRPVRQPGKTFATMDHNVSTQTKDINACGEMARIQMQELIKNCKEFGVELYDLNHPYQGIVHVMGPEQGVTLPGMTIVCGDSHTATHGAFGALAFGIGTSEVEHVLATQTLKQGRAKTMKIEVQGKAAPGITAKDIVLAIIGKTGSAGGTGHVVEFCGEAIRDLSMEGRMTLCNMAIEMGAKAGLVAPDETTFNYVKGRLHAPKGKDFDDAVAYWKTLQTDEGATFDTVVTLQAEEISPQVTWGTNPGQVISVNDNIPDPASFADPVERASAEKALAYMGLKPGIPLTEVAIDKVFIGSCTNSRIEDLRAAAEIAKGRKVAPGVQALVVPGSGPVKAQAEAEGLDKIFIEAGFEWRLPGCSMCGAMNNDRLNPGERCASTSNRNFEGRQGRGGRTHLVSPAMAAAAAVTGHFADIRNIK

SEQ ID NO: 10 - protein, 466 aa, Artificial Sequence
  Synthesized - Modified LeuC (V35A L411V)
MAKTLYEKLFDAHVVYEAENETPLLYIDRHLVHEATSPQAFDGLRAHGRPVRQPGKTFATMDHNVSTQTKDINACGEMARIQMQELIKNCKEFGVELYDLNHPYQGIVHVMGPEQGVTLPGMTIVCGDSHTATHGAFGALAFGIGTSEVEHVLATQTLKQGRAKTMKIEVQGKAAPGITAKDIVLAIIGKTGSAGGTGHVVEFCGEAIRDLSMEGRMTLCNMAIEMGAKAGLVAPDETTFNYVKGRLHAPKGKDFDDAVAYWKTLQTDEGATFDTVVTLQAEEISPQVTWGTNPGQVISVNDNIPDPASFADPVERASAEKALAYMGLKPGIPLTEVAIDKVFIGSCTNSRIEDLRAAAEIAKGRKVAPGVQALVVPGSGPVKAQAEAEGLDKIFIEAGFEWRLPGCSMCVAMNNDRLNPGERCASTSNRNFEGRQGRGGRTHLVSPAMAAAAAVTGHFADIRNIK

SEQ ID NO: 11 - protein, 466 aa, Artificial Sequence
  Synthesized - Modified LeuC (V35G L411A)
MAKTLYEKLFDAHVVYEAENETPLLYIDRHLVHEGTSPQAFDGLRAHGRPVRQPGKTFATMDHNVSTQTKDINACGEMARIQMQELIKNCKEFGVELYDLNHPYQGIVHVMGPEQGVTLPGMTIVCGDSHTATHGAFGALAFGIGTSEVEHVLATQTLKQGRAKTMKIEVQGKAAPGITAKDIVLAIIGKTGSAGGTGHVVEFCGEAIRDLSMEGRMTLCNMAIEMGAKAGLVAPDETTFNYVKGRLHAPKGKDFDDAVAYWKTLQTDEGATFDTVVTLQAEEISPQVTWGTNPGQVISVNDNIPDPASFADPVERASAEKALAYMGLKPGIPLTEVAIDKVFIGSCTNSRIEDLRAAAEIAKGRKVAPGVQALVVPGSGPVKAQAEAEGLDKIFIEAGFEWRLPGCSMCAAMNNDRLNPGERCASTSNRNFEGRQGRGGRTHLVSPAMAAAAAVTGHFADIRNIK

SEQ ID NO: 12 - protein, 466 aa, Artificial Sequence
  Synthesized - Modified LeuC (V35G L411G)
MAKTLYEKLFDAHVVYEAENETPLLYIDRHLVHEGTSPQAFDGLRAHGRPVRQPGKTFATMDHNVSTQTKDINACGEMARIQMQELIKNCKEFGVELYDLNHPYQGIVHVMGPEQGVTLPGMTIVCGDSHTATHGAFGALAFGIGTSEVEHVLATQTLKQGRAKTMKIEVQGKAAPGITAKDIVLAIIGKTGSAGGTGHVVEFCGEAIRDLSMEGRMTLCNMAIEMGAKAGLVAPDETTFNYVKGRLHAPKGKDFDDAVAYWKTLQTDEGATFDTVVTLQAEEISPQVTWGTNPGQVISVNDNIPDPASFADPVERASAEKALAYMGLKPGIPLTEVAIDKVFIGSCTNSRIEDLRAAAEIAKGRKVAPGVQALVVPGSGPVKAQAEAEGLDKIFIEAGFEWRLPGCSMCGAMNNDRLNPGERCASTSNRNFEGRQGRGGRTHLVSPAMAAAAAVTGHFADIRNIK

SEQ ID NO: 13 - protein, 466 aa, Artificial Sequence
  Synthesized - Modified LeuC (V35G L411V)
MAKTLYEKLFDAHVVYEAENETPLLYIDRHLVHEGTSPQAFDGLRAHGRPVRQPGKTFATMDHNVSTQTKDINACGEMARIQMQELIKNCKEFGVELYDLNHPYQGIVHVMGPEQGVTLPGMTIVCGDSHTATHGAFGALAFGIGTSEVEHVLATQTLKQGRAKTMKIEVQGKAAPGITAKDIVLAIIGKTGSAGGTGHVVEFCGEAIRDLSMEGRMTLCNMAIEMGAKAGLVAPDETTFNYVKGRLHAPKGKDFDDAVAYWKTLQTDEGATFDTVVTLQAEEISPQVTWGTNPGQVISVNDNIPDPASFADPVERASAEKALAYMGLKPGIPLTEVAIDKVFIGSCTNSRIEDLRAAAEIAKGRKVAPGVQALVVPGSGPVKAQAEAEGLDKIFIEAGFEWRLPGCSMCVAMNNDRLNPGERCASTSNRNFEGRQGRGGRTHLVSPAMAAAAAVTGHFADIRNIK

SEQ ID NO: 14 - protein, 201 aa, Artificial Sequence
  Synthesized - Modified LeuD (H88A)
MAEKFIKHTGLVVPLDAANVDTDAIIPKQFLQKVTRTGFGAHLFNDWRFLDEKGQQPNPDFVLNFPQYQGASILLARENFGCGSSREAAPWALTDYGFKVVIAPSFADIFYGNSFNNQLLPVKLSDAEVDELFALVKANPGIHFDVDLEAQEVKAGEKTYRFTIDAFRRHCMMNGLDSIGLTLQHDDAIAAYEAKQPAFMN

SEQ ID NO: 15 - protein, 201 aa, Artificial Sequence
  Synthesized - Modified LeuD (H88G)
MAEKFIKHTGLVVPLDAANVDTDAIIPKQFLQKVTRTGFGAHLFNDWRFLDEKGQQPNPDFVLNFPQYQGASILLARENFGCGSSREGAPWALTDYGFKVVIAPSFADIFYGNSFNNQLLPVKLSDAEVDELFALVKANPGIHFDVDLEAQEVKAGEKTYRFTIDAFRRHCMMNGLDSIGLTLQHDDAIAAYEAKQPAFMN

SEQ ID NO: 16 - protein, 201 aa, Artificial Sequence
  Synthesized - Modified LeuD (H88V)
MAEKFIKHTGLVVPLDAANVDTDAIIPKQFLQKVTRTGFGAHLFNDWRFLDEKGQQPNPDFVLNFPQYQGASILLARENFGCGSSREVAPWALTDYGFKVVIAPSFADIFYGNSFNNQLLPVKLSDAEVDELFALVKANPGIHFDVDLEAQEVKAGEKTYRFTIDAFRRHCMMNGLDSIGLTLQHDDAIAAYEAKQPAFMN

SEQ ID NO: 17 - protein, 201 aa, Artificial Sequence
  Synthesized - Modified LeuD (H88S)
MAEKFIKHTGLVVPLDAANVDTDAIIPKQFLQKVTRTGFGAHLFNDWRFLDEKGQQPNPDFVLNFPQYQGASILLARENFGCGSSRESAPWALTDYGFKVVIAPSFADIFYGNSFNNQLLPVKLSDAEVDELFALVKANPGIHFDVDLEAQEVKAGEKTYRFTIDAFRRHCMMNGLDSIGLTLQHDDAIAAYEAKQPAFMN

SEQ ID NO: 18 - protein, 201 aa, Artificial Sequence
  Synthesized - Modified LeuD (L31A)
MAEKFIKHTGLVVPLDAANVDTDAIIPKQFAQKVTRTGFGAHLFNDWRFLDEKGQQPNPDFVLNFPQYQGASILLARENFGCGSSREHAPWALTDYGFKVVIAPSFADIFYGNSFNNQLLPVKLSDAEVDELFALVKANPGIHFDVDLEAQEVKAGEKTYRFTIDAFRRHCMMNGLDSIGLTLQHDDAIAAYEAKQPAFMN

SEQ ID NO: 19 - protein, 201 aa, Artificial Sequence
  Synthesized - Modified LeuD (L31A H88A)
MAEKFIKHTGLVVPLDAANVDTDAIIPKQFAQKVTRTGFGAHLFNDWRFLDEKGQQPNPDFVLNFPQYQGASILLARENFGCGSSREAAPWALTDYGFKVVIAPSFADIFYGNSFNNQLLPVKLSDAEVDELFALVKANPGIHFDVDLEAQEVKAGEKTYRFTIDAFRRHCMMNGLDSIGLTLQHDDAIAAYEAKQPAFMN

SEQ ID NO: 20 - protein, 201 aa, Artificial Sequence
  Synthesized - Modified LeuD (L31A H88G)
MAEKFIKHTGLVVPLDAANVDTDAIIPKQFAQKVTRTGFGAHLFNDWRFLDEKGQQPNPDFVLNFPQYQGASILLARENFGCGSSREGAPWALTDYGFKVVIAPSFADIFYGNSFNNQLLPVKLSDAEVDELFALVKANPGIHFDVDLEAQEVKAGEKTYRFTIDAFRRHCMMNGLDSIGLTLQHDDAIAAYEAKQPAFMN

SEQ ID NO: 21 - protein, 201 aa, Artificial Sequence
  Synthesized - Modified LeuD (L31A H88V)
MAEKFIKHTGLVVPLDAANVDTDAIIPKQFAQKVTRTGFGAHLFNDWRFLDEKGQQPNPDFVLNFPQYQGASILLARENFGCGSSREVAPWALTDYGFKVVIAPSFADIFYGNSFNNQLLPVKLSDAEVDELFALVKANPGIHFDVDLEAQEVKAGEKTYRFTIDAFRRHCMMNGLDSIGLTLQHDDAIAAYEAKQPAFMN

SEQ ID NO: 22 - protein, 201 aa, Artificial Sequence
  Synthesized - Modified LeuD (L31A H88S)
MAEKFIKHTGLVVPLDAANVDTDAIIPKQFAQKVTRTGFGAHLFNDWRFLDEKGQQPNPDFVLNFPQYQGASILLARENFGCGSSRESAPWALTDYGFKVVIAPSFADIFYGNSFNNQLLPVKLSDAEVDELFALVKANPGIHFDVDLEAQEVKAGEKTYRFTIDAFRRHCMMNGLDSIGLTLQHDDAIAAYEAKQPAFMN

SEQ ID NO: 23 - protein, 201 aa, Artificial Sequence
  Synthesized - Modified LeuD (L31G)
MAEKFIKHTGLVVPLDAANVDTDAIIPKQFGQKVTRTGFGAHLFNDWRFLDEKGQQPNPDFVLNFPQYQGASILLARENFGCGSSREHAPWALTDYGFKVVIAPSFADIFYGNSFNNQLLPVKLSDAEVDELFALVKANPGIHFDVDLEAQEVKAGEKTYRFTIDAFRRHCMMNGLDSIGLTLQHDDAIAAYEAKQPAFMN

SEQ ID NO: 24 - protein, 201 aa, Artificial Sequence
  Synthesized - Modified LeuD (L31G H88A)
MAEKFIKHTGLVVPLDAANVDTDAIIPKQFGQKVTRTGFGAHLFNDWRFLDEKGQQPNPDFVLNFPQYQGASILLARENFGCGSSREAAPWALTDYGFKVVIAPSFADIFYGNSFNNQLLPVKLSDAEVDELFALVKANPGIHFDVDLEAQEVKAGEKTYRFTIDAFRRHCMMNGLDSIGLTLQHDDAIAAYEAKQPAFMN

SEQ ID NO: 25 - protein, 201 aa, Artificial Sequence
  Synthesized - Modified LeuD (L31G H88G)
MAEKFIKHTGLVVPLDAANVDTDAIIPKQFGQKVTRTGFGAHLFNDWRFLDEKGQQPNPDFVLNFPQYQGASILLARENFGCGSSREGAPWALTDYGFKVVIAPSFADIFYGNSFNNQLLPVKLSDAEVDELFALVKANPGIHFDVDLEAQEVKAGEKTYRFTIDAFRRHCMMNGLDSIGLTLQHDDAIAAYEAKQPAFMN

SEQ ID NO: 26 - protein, 201 aa, Artificial Sequence
  Synthesized - Modified LeuD (L31G H88V)
MAEKFIKHTGLVVPLDAANVDTDAIIPKQFGQKVTRTGFGAHLFNDWRFLDEKGQQPNPDFVLNFPQYQGASILLARENFGCGSSREVAPWALTDYGFKVVIAPSFADIFYGNSFNNQLLPVKLSDAEVDELFALVKANPGIHFDVDLEAQEVKAGEKTYRFTIDAFRRHCMMNGLDSIGLTLQHDDAIAAYEAKQPAFMN

SEQ ID NO: 27 - protein, 201 aa, Artificial Sequence
  Synthesized - Modified LeuD( L31G H88S)
MAEKFIKHTGLVVPLDAANVDTDAIIPKQFGQKVTRTGFGAHLFNDWRFLDEKGQQPNPDFVLNFPQYQGASILLARENFGCGSSRESAPWALTDYGFKVVIAPSFADIFYGNSFNNQLLPVKLSDAEVDELFALVKANPGIHFDVDLEAQEVKAGEKTYRFTIDAFRRHCMMNGLDSIGLTLQHDDAIAAYEAKQPAFMN

SEQ ID NO: 28 - protein, 201 aa, Artificial Sequence
  Synthesized - Modified LeuD (L31V)
MAEKFIKHTGLVVPLDAANVDTDAIIPKQFVQKVTRTGFGAHLFNDWRFLDEKGQQPNPDFVLNFPQYQGASILLARENFGCGSSREHAPWALTDYGFKVVIAPSFADIFYGNSFNNQLLPVKLSDAEVDELFALVKANPGIHFDVDLEAQEVKAGEKTYRFTIDAFRRHCMMNGLDSIGLTLQHDDAIAAYEAKQPAFMN

SEQ ID NO: 29 - protein, 201 aa, Artificial Sequence
  Synthesized - Modified LeuD (L31V H88A)
MAEKFIKHTGLVVPLDAANVDTDAIIPKQFVQKVTRTGFGAHLFNDWRFLDEKGQQPNPDFVLNFPQYQGASILLARENFGCGSSREAAPWALTDYGFKVVIAPSFADIFYGNSFNNQLLPVKLSDAEVDELFALVKANPGIHFDVDLEAQEVKAGEKTYRFTIDAFRRHCMMNGLDSIGLTLQHDDAIAAYEAKQPAFMN

SEQ ID NO: 30 - protein, 201 aa, Artificial Sequence
  Synthesized - Modified LeuD (L31V H88G)
MAEKFIKHTGLVVPLDAANVDTDAIIPKQFVQKVTRTGFGAHLFNDWRFLDEKGQQPNPDFVLNFPQYQGASILLARENFGCGSSREGAPWALTDYGFKVVIAPSFADIFYGNSFNNQLLPVKLSDAEVDELFALVKANPGIHFDVDLEAQEVKAGEKTYRFTIDAFRRHCMMNGLDSIGLTLQHDDAIAAYEAKQPAFMN

SEQ ID NO: 31 - protein, 201 aa, Artificial Sequence
  Synthesized - Modified LeuD (L31V H88V)
MAEKFIKHTGLVVPLDAANVDTDAIIPKQFVQKVTRTGFGAHLFNDWRFLDEKGQQPNPDFVLNFPQYQGASILLARENFGCGSSREVAPWALTDYGFKVVIAPSFADIFYGNSFNNQLLPVKLSDAEVDELFALVKANPGIHFDVDLEAQEVKAGEKTYRFTIDAFRRHCMMNGLDSIGLTLQHDDAIAAYEAKQPAFMN

SEQ ID NO: 32 - protein, 201 aa, Artificial Sequence
  Synthesized - Modified LeuD (L31V H88S)
MAEKFIKHTGLVVPLDAANVDTDAIIPKQFVQKVTRTGFGAHLFNDWRFLDEKGQQPNPDFVLNFPQYQGASILLARENFGCGSSRESAPWALTDYGFKVVIAPSFADIFYGNSFNNQLLPVKLSDAEVDELFALVKANPGIHFDVDLEAQEVKAGEKTYRFTIDAFRRHCMMNGLDSIGLTLQHDDAIAAYEAKQPAFMN

SEQ ID NO: 33 - protein, 201 aa, Artificial Sequence
  Synthesized - Modified LeuD (L31S)
MAEKFIKHTGLVVPLDAANVDTDAIIPKQFSQKVTRTGFGAHLFNDWRFLDEKGQQPNPDFVLNFPQYQGASILLARENFGCGSSREHAPWALTDYGFKVVIAPSFADIFYGNSFNNQLLPVKLSDAEVDELFALVKANPGIHFDVDLEAQEVKAGEKTYRFTIDAFRRHCMMNGLDSIGLTLQHDDAIAAYEAKQPAFMN

SEQ ID NO: 34 - protein, 201 aa, Artificial Sequence
  Synthesized - Modified LeuD (L31S H88A)
MAEKFIKHTGLVVPLDAANVDTDAIIPKQFSQKVTRTGFGAHLFNDWRFLDEKGQQPNPDFVLNFPQYQGASILLARENFGCGSSREAAPWALTDYGFKVVIAPSFADIFYGNSFNNQLLPVKLSDAEVDELFALVKANPGIHFDVDLEAQEVKAGEKTYRFTIDAFRRHCMMNGLDSIGLTLQHDDAIAAYEAKQPAFMN

SEQ ID NO: 35 - protein, 201 aa, Artificial Sequence
  Synthesized - Modified LeuD (L31S H88G)
MAEKFIKHTGLVVPLDAANVDTDAIIPKQFSQKVTRTGFGAHLFNDWRFLDEKGQQPNPDFVLNFPQYQGASILLARENFGCGSSREGAPWALTDYGFKVVIAPSFADIFYGNSFNNQLLPVKLSDAEVDELFALVKANPGIHFDVDLEAQEVKAGEKTYRFTIDAFRRHCMMNGLDSIGLTLQHDDAIAAYEAKQPAFMN

SEQ ID NO: 36 - protein, 201 aa, Artificial Sequence
  Synthesized - Modified LeuD (L31S H88V)
MAEKFIKHTGLVVPLDAANVDTDAIIPKQFSQKVTRTGFGAHLFNDWRFLDEKGQQPNPDFVLNFPQYQGASILLARENFGCGSSREVAPWALTDYGFKVVIAPSFADIFYGNSFNNQLLPVKLSDAEVDELFALVKANPGIHFDVDLEAQEVKAGEKTYRFTIDAFRRHCMMNGLDSIGLTLQHDDAIAAYEAKQPAFMN

SEQ ID NO: 37 - protein, 201 aa, Artificial Sequence
  Synthesized - Modified LeuD (L31S H88S)
MAEKFIKHTGLVVPLDAANVDTDAIIPKQFSQKVTRTGFGAHLFNDWRFLDEKGQQPNPDFVLNFPQYQGASILLARENFGCGSSRESAPWALTDYGFKVVIAPSFADIFYGNSFNNQLLPVKLSDAEVDELFALVKANPGIHFDVDLEAQEVKAGEKTYRFTIDAFRRHCMMNGLDSIGLTLQHDDAIAAYEAKQPAFMN